European Patent Application EP 4 793 369 A1, published August 19, 2026. Title: Gemin4基因及Gemin4蛋白在肿瘤中的应用. Applicant: 南京安吉生物科技有限公司. Application CN. The sequence listing filed with the application follows.

SEQUENCE LISTING (8 sequences)

SEQ ID NO: 1 - DNA, 3177 bp, synthetic construct
  source 1..3177: mol_type = other DNA
atggacctaggacccttgaacatctgtgaagaaatgactattctgcatggaggcttcttgctggccgagcagctgttccaccctaaggcactggcagaattaacaaagtctgactgggaacgtgttggacggcccatcgtggaggccttaagggagatctcctcggctgcagcacactcccagccctttgcctggaagaagaaagccctgatcatcatctgggccaaggttctgcagccgcaccccgtgaccccgtccgacacagagacacggtggcaggaagacctgttcttctcggtgggcaacatgatccccaccatcaaccacaccatcctcttcgagctgctcaaatccctggaagcttctggactctttatccagctcctgatggccctgcccaccaccatctgccatgcagaactagagcgctttctggaacatgtgaccgttgacacttctgccgaagacgtggccttcttcctggacgtctggtgggaggtgatgaagcacaagggtcacccgcaggaccccctgctctcccagtttagtgcaatggcccataagtacctgcctgccttagatgagttcccccatcctccaaagaggcttaggtcagacccagacgcgtgccccaccatgcccctgttggccatgctgctccgcgggctgacacagatccagagtcggatcctgggcccggggaggaagtgctgtgcgctggccaacctggctgacatgctgactgtgtttgcgctgacagaggacgacccccaggaggtgtctgcaaccgtgtatctggacaaactggccacggtgatctctgtgtggaactcggacacccagaatccctaccaccagcaggcgctggcagagaaggtgaaggaggcagaacgggatgtcagcctgacctcgctggccaaactccccagtgagaccattttcgtgggctgcgagttcctgcaccacctgctgcgggagtggggggaggagttgcaggccgtgctccgcagcagccaggggacaagttacgacagctaccggctgtgcgacagtctgacttccttcagccagaacgcgacgctctacctgaaccgcaccagcctgtccaaggaggacaggcaggtggtctctgagctggcggagtgtgtcagggacttcctgaggaaaacgagcacggtgctgaagaacagggccttggaggatatcacagcttccattgccatggccgtcatccagcagaagatggaccgccatatggaagtgtgctacatttttgcctctgagaagaagtgggccttctcggacgagtgggtagcctgcctggggagtaacagggccctcttccgacagccagacttggtgttgaggctgctggaaacagtgatagacgtcagcacagctgacagagccatccctgagtctcagatccggcaggtgatccacctgatcctggaatgttacgcagacctctccctgccaggtaaaaataaagtccttgcaggtatcctgcgttcctgggggcgaaagggcctctctgaaaagttgctggcttatgtggagggttttcaggaagacctcaatacaacttttaaccagctcactcagagtgcctccgaacagggcttggcaaaagctgtggcctccgtggcccgcctggtcatagtgcacccggaagtcacggtgaagaaaatgtgcagcctggctgtggtcaatctcggcacccacaagttcctggcccagattctcactgccttccctgcccttaggtttgtggaagagcagggtcccaattcatctgccactttcatggtgtcatgcctcaaagaaaccgtctggatgaagttctctacacccaaggaagaaaagcaatttttagagctcctgaactgcctgatgagtcccgtgaaaccccaagggattccagtggctgctcttcttgagccagacgaggtgctgaaggaatttgtcctgcctttcttgaggttagatgttgaagaggtagacctcagtctgaggatcttcatccagactctagaggcaaacgcgtgccgagaggaatactggctccagacctgctccccgtttccactcctcttcagcttgtgccagctcttggaccgcttcagcaaatactggcagcttcccaaggagaagcggtgcctctctttggataggaaggatctagcgatccatatcctggagctcctgtgtgagattgtatcagccaatgctgagaccttctccccggatgtctggatcaagtccctgtcctggctccaccgcaagttagaacagctagactggactgtgggcctgaggctgaagagcttcttcgaggggcacttcaagtgtgaagtgccagccacactttttgagatctgtaagctttcagaagacgagtggacctcccaggcccacccagggtacggggctggcacggggctcctggcctggatggagtgctgctgcgtctccagcggcatctcggagaggatgctgtctctcttggtggtggacgtgggcaatcctgaggaggtcagactgttcagcaaaggctttctggtggccctggtgcaagtcatgccttggtgcagccctcaggagtggcagcgccttcaccagctgaccaggagactgctggagaagcagctcctccatgtcccttatagcctggaatatattcagtttgttcccctgctcaacctgaagccctttgcccaggagttgcaactctccgtcctcttcctgaggactttccagtttctctgcagccatagctgtcgtgattggcttcctctggaaggctggaaccacgtggtcaaactcctctgtggcagtctgacccgcctcctggactcagtcagggcgatacaggcagctggcccttgggttcaaggaccagagcaggacctgacccaggaagccctgtttgtttacacccaggtgttctgccatgctctgcacatcatggccatgctccacccggaggtctgtgagccactctacgttttagccttggaaaccctcacctgctatgagactttgagcaagaccaacccttctgtcagctccttgctccagagggcacacgagcagcgcttcttaaagtccattgctgagggcatcggccctgaagaacggcgccaaaccctgttgcagaagatgagcagcttctga

SEQ ID NO: 2 - protein, 1058 aa, synthetic construct
MDLGPLNICEEMTILHGGFLLAEQLFHPKALAELTKSDWERVGRPIVEALREISSAAAHSQPFAWKKKALIIIWAKVLQPHPVTPSDTETRWQEDLFFSVGNMIPTINHTILFELLKSLEASGLFIQLLMALPTTICHAELERFLEHVTVDTSAEDVAFFLDVWWEVMKHKGHPQDPLLSQFSAMAHKYLPALDEFPHPPKRLRSDPDACPTMPLLAMLLRGLTQIQSRILGPGRKCCALANLADMLTVFALTEDDPQEVSATVYLDKLATVISVWNSDTQNPYHQQALAEKVKEAERDVSLTSLAKLPSETIFVGCEFLHHLLREWGEELQAVLRSSQGTSYDSYRLCDSLTSFSQNATLYLNRTSLSKEDRQVVSELAECVRDFLRKTSTVLKNRALEDITASIAMAVIQQKMDRHMEVCYIFASEKKWAFSDEWVACLGSNRALFRQPDLVLRLLETVIDVSTADRAIPESQIRQVIHLILECYADLSLPGKNKVLAGILRSWGRKGLSEKLLAYVEGFQEDLNTTFNQLTQSASEQGLAKAVASVARLVIVHPEVTVKKMCSLAVVNLGTHKFLAQILTAFPALRFVEEQGPNSSATFMVSCLKETVWMKFSTPKEEKQFLELLNCLMSPVKPQGIPVAALLEPDEVLKEFVLPFLRLDVEEVDLSLRIFIQTLEANACREEYWLQTCSPFPLLFSLCQLLDRFSKYWQLPKEKRCLSLDRKDLAIHILELLCEIVSANAETFSPDVWIKSLSWLHRKLEQLDWTVGLRLKSFFEGHFKCEVPATLFEICKLSEDEWTSQAHPGYGAGTGLLAWMECCCVSSGISERMLSLLVVDVGNPEEVRLFSKGFLVALVQVMPWCSPQEWQRLHQLTRRLLEKQLLHVPYSLEYIQFVPLLNLKPFAQELQLSVLFLRTFQFLCSHSCRDWLPLEGWNHVVKLLCGSLTRLLDSVRAIQAAGPWVQGPEQDLTQEALFVYTQVFCHALHIMAMLHPEVCEPLYVLALETLTCYETLSKTNPSVSSLLQRAHEQRFLKSIAEGIGPEERRQTLLQKMSSF

SEQ ID NO: 3 - DNA, 20 bp, synthetic construct
  source 1..20: mol_type = other DNA
cctcacctgctatgagactt

SEQ ID NO: 4 - DNA, 20 bp, synthetic construct
  source 1..20: mol_type = other DNA
gccctcagcaatggacttta

SEQ ID NO: 5 - RNA, 21 nt, synthetic construct
  source 1..21: mol_type = other RNA
gctcctgtgtgagattgtatt

SEQ ID NO: 6 - DNA, 20 bp, synthetic construct
  source 1..20: mol_type = other DNA
tgcaccaccaactgcttagc

SEQ ID NO: 7 - DNA, 21 bp, synthetic construct
  source 1..21: mol_type = other DNA
ggcatggactgtggtcatgag

SEQ ID NO: 8 - RNA, 21 nt, synthetic construct
  source 1..21: mol_type = other RNA
acgtgacacgttcggagaatt